European Patent Specification EP 4 200 018 B1, published January 1, 2025. Title: ANTI-PAR-2 ANTIBODIES AND METHODS OF USE THEREOF. Applicant: CEPHALON, INC. BRACKEN, ANNA MIKAELA CLARKE, ADAM COOKSEY, BRIDGET A. DOYLE, ANTHONY GERARD LIDDAMENT, MARK TERENCE POLLARD, MATTHEW POULTON, LYNN QUIGLEY, ANNA MARIA MATILDA ROZENFELD, JULIA SZABAT, MARTA. The sequence listing filed with the application follows.

SEQUENCE LISTING (162 sequences)

SEQ ID NO: 1 - protein, 10 aa, artificial sequence
  VH CDR1
  misc_feature (5)..(5): Wherein Xaa is Asp or Ser
  misc_feature (6)..(6): Wherein Xaa is Ser or Tyr
  misc_feature (8)..(8): Wherein Xaa is Gly or Ala
  misc_feature (9)..(9): Wherein Xaa is Val, Gly, or Isoleucine,
  misc_feature (10)..(10): Wherein Xaa is IIe or Ser
GFSLXXYXXX

SEQ ID NO: 2 - protein, 11 aa, artificial sequence
  VH CDR2
  misc_feature (6)..(6): Wherein Xaa is Gly or Glu
  misc_feature (8)..(8): Wherein Xaa is Val or Thr
  misc_feature (11)..(11): Wherein Xaa is Asn, Ala, Gly, or Tyr
VIWGNXNXYYX

SEQ ID NO: 3 - protein, 11 aa, artificial sequence
  VH CDR3
  misc_Feature (2)..(2): Wherein Xaa is Arg or Lys
  misc_Feature (4)..(4): Wherein Xaa is Tyr, Trp, or Phe
  misc_Feature (7)..(7): Wherein Xaa is Tyr or His
WXGXKDXPFDY

SEQ ID NO: 4 - protein, 11 aa, artificial sequence
  VL CDR1
  misc_feature (1)..(1): Wherein Xaa is Lys or Arg
  misc_feature (6)..(6): Wherein Xaa is Ile or Val
  misc_feature (9)..(9): Wherein Xaa is Tyr, Trp or Phe
XASQNXYKXLD

SEQ ID NO: 5 - protein, 7 aa, artificial sequence
  VL CDR2
  misc_feature (1)..(1): Wherein Xaa is Asn or Asp
  misc_feature (2)..(2): Wherein Xaa is Thr or Ala
  misc_feature (3)..(3): Wherein Xaa is Asn, Ser, or Tyr
  misc_feature (4)..(4): Wherein Xaa is Ser, Thr, or Asn
  misc_feature (5)..(5): Wherein Xaa is Leu or Arg
  misc_feature (6)..(6): Wherein Xaa is His or Ala
XXXXXXT

SEQ ID NO: 6 - protein, 8 aa, artificial sequence
  VL CDR3
  misc_feature (1)..(1): wherein Xaa is Leu or Glu
  misc_feature (4)..(4): wherein Xaa is Asn, Gly or His
  misc_feature (5)..(5): wherein Xaa is Ser or His
XQHXXGWT

SEQ ID NO: 7 - protein, 10 aa, artificial sequence
  Anti-PAR-2 (309) Heavy Chain CDR1
GFSLNSYGVI

SEQ ID NO: 8 - protein, 11 aa, artificial sequence
  Anti-PAR-2 (309) Heavy Chain CDR2
VIWGNGNTYYN

SEQ ID NO: 9 - protein, 11 aa, artificial sequence
  Anti-PAR-2 (309 and 309-4e) Heavy Chain CDR3
WRGYKDYPFDY

SEQ ID NO: 10 - protein, 10 aa, artificial sequence
  Anti-PAR-2 (P24E1102, P24E976, P24E1099, and P24E1103) Heavy Chain CDR1
GFSLSSYAIS

SEQ ID NO: 11 - protein, 11 aa, artificial sequence
  Anti-PAR-2 (P24E1102, P24E976, P24E1099, and P24E1103) Heavy Chain CDR2
VIWGNQNVYYA

SEQ ID NO: 12 - protein, 11 aa, artificial sequence
  Anti-PAR-2 (P24E1102, P24E976, P24E1099, and P24E1103) Heavy Chain CDR3
WKGYKDYPFDY

SEQ ID NO: 13 - protein, 11 aa, artificial sequence
  Anti-PAR-2 (309 and 309-4e) Light Chain CDR1
KASQNIYKYLD

SEQ ID NO: 14 - protein, 7 aa, artificial sequence
  Anti-PAR-2 (309 and 309-4e) Light Chain CDR2
NTNSLHT

SEQ ID NO: 15 - protein, 8 aa, artificial sequence
  Anti-PAR-2 (309 and 309-4e) Light Chain CDR3
LQHNSGWT

SEQ ID NO: 16 - protein, 11 aa, artificial sequence
  Anti-PAR-2 (P24E1102, P24E976, P24E1099, and P24E1103) Light Chain CDR1
RASQNVYKWLD

SEQ ID NO: 17 - protein, 7 aa, artificial sequence
  Anti-PAR-2 (P24E1102) Light Chain CDR2
NANTRAT

SEQ ID NO: 18 - protein, 8 aa, artificial sequence
  Anti-PAR-2 (P24E1102, P24E976, P24E1099, and P24E1103) Light Chain CDR3
QQHHSGWT

SEQ ID NO: 19 - protein, 7 aa, artificial sequence
  Anti-PAR-2 (P24E976) Light Chain CDR2
NAYSRAT

SEQ ID NO: 20 - protein, 119 aa, artificial sequence
  Anti-PAR-2 (309-4e) Variable Heavy Chain sequence
QVQLVQSGAEVKKPGSSVKVSCKASGFSLNSYGVIWVRQAPGQGLEWMGVIWGNGNTYYNQKFQGRVTITADESTSTAYMELSSLRSEDTAVYYCARWRGYKDYPFDYWGQGTLVTVSS

SEQ ID NO: 21 - protein, 119 aa, artificial sequence
  Anti-PAR-2 (P24E1102, P24E976, P24E1099, and P24E1103) Variable Heavy Chain sequence
QVQLVQSGAEVKKPGSSVKVSCKASGFSLSSYAISWVRQAPGQGLEWMGVIWGNQNVYYAQKFQGRVTITADESTSTAYMELSSLRSEDTAVYYCARWKGYKDYPFDYWGQGTLVTVSS

SEQ ID NO: 22 - protein, 7 aa, artificial sequence
  Anti-PAR-2 (P24E1103) Light Chain CDR2
NANNRAT

SEQ ID NO: 23 - protein, 106 aa, artificial sequence
  Anti-PAR-2 (309-4e) Variable Light Chain Sequence
EIVLTQSPATLSLSPGERATLSCKASQNIYKYLDWYQQKPGQAPRLLIYNTNSLHTGIPARFSGSGSGRDFTLTISSLEPEDFAVYYCLQHNSGWTFGGGTKVEIK

SEQ ID NO: 24 - protein, 106 aa, artificial sequence
  Anti-PAR-2 (P24E1102) Variable Light Chain Sequence
EIVLTQSPATLSLSPGERATLSCRASQNVYKWLDWYQQKPGQAPRLLIYNANTRATGIPARFSGSGSGRDFTLTISSLEPEDFAVYYCQQHHSGWTFGGGTKVEIK

SEQ ID NO: 25 - protein, 106 aa, artificial sequence
  Anti-PAR-2 (P24E976) Light Chain Sequence
EIVLTQSPATLSLSPGERATLSCRASQNVYKWLDWYQQKPGQAPRLLIYNAYSRATGIPARFSGSGSGRDFTLTISSLEPEDFAVYYCQQHHSGWTFGGGTKVEIK

SEQ ID NO: 26 - protein, 106 aa, artificial sequence
  Anti-PAR-2 (P24E1099) Variable Light Chain Sequence
EIVLTQSPATLSLSPGERATLSCRASQNVYKWLDWYQQKPGQAPRLLIYNANSRATGIPARFSGSGSGRDFTLTISSLEPEDFAVYYCQQHHSGWTFGGGTKVEIK

SEQ ID NO: 27 - protein, 106 aa, artificial sequence
  Anti-PAR-2 (P24E1103) Variable Light Chain Sequence
EIVLTQSPATLSLSPGERATLSCRASQNVYKWLDWYQQKPGQAPRLLIYNANNRATGIPARFSGSGSGRDFTLTISSLEPEDFAVYYCQQHHSGWTFGGGTKVEIK

SEQ ID NO: 28 - protein, 397 aa, artificial sequence
  human PAR-2
MRSPSAAWLLGAAILLAASLSCSGTIQGTNRSSKGRSLIGKVDGTSHVTGKGVTVETVFSVDEFSASVLTGKLTTVFLPIVYTIVFVVGLPSNGMALWVFLFRTKKKHPAVIYMANLALADLLSVIWFPLKIAYHIHGNNWIYGEALCNVLIGFFYGNMYCSILFMTCLSVQRYWVIVNPMGHSRKKANIAIGISLAIWLLILLVTIPLYVVKQTIFIPALNITTCHDVLPEQLLVGDMFNYFLSLAIGVFLFPAFLTASAYVLMIRMLRSSAMDENSEKKRKRAIKLIVTVLAMYLICFTPSNLLLVVHYFLIKSQGQSHVYALYIVALCLSTLNSCIDPFVYYFVSHDFRDHAKNALLCRSVRTVKQMQVSLTSKKHSRKSSSYSSSSTTVKTSY

SEQ ID NO: 29 - protein, 7 aa, artificial sequence
  Anti-PAR-2 ("P24E1099") Light Chain CDR2
NANSRAT

SEQ ID NO: 30 - protein, 438 aa, artificial sequence
  Cynomolgus monkey PAR-2
  misc_feature (406)..(406): Xaa can be any naturally occurring amino acid
LGHLVLTHLLVALFGMGSWAAVNGIWVELPVVVKDLPEGWSLPSYLSVIVALGNLGLLVVTLWRRLAPGKGERVPIQVVQVLSVVGTALLAPLWHHVAPVAGQLHSVAFLTLALVLALACCTSNVTFLPFLSHLPPPFLRSFFLGQGLSALLPCVLALVQGVGRLECSPAPTNGTSGPPLNFPERFPASTFFWALTALLVTSAAAFQGLLLLLPSLPSVTTGGAGPELPLGSPGAEEEEKEEEEALPLQEPPSQAAGTIPGPDPEAHQLFSAHGAFLLGLLAITSALTNGVLPAVQSFSCLPYGRLAYHLAVVLGSAANPLACFLAMGVLCRSLAGLVGLSLLGMLFGAYLMVLAILSPCPPLVGTTAGVVLVVLSWVLCLCVFSYVKVAASSLLHGGGRPALLAXGVAIQVGSLLGAGTMFPPTSIYHVFQSRKDCV

SEQ ID NO: 31 - protein, 418 aa, artificial sequence
  Cynomolgus monkey PAR-2 (without the signal sequence)
  misc_feature (386)..(386): Xaa can be any naturally occurring amino acid
AVNGIWVELPVVVKDLPEGWSLPSYLSVIVALGNLGLLVVTLWRRLAPGKGERVPIQVVQVLSVVGTALLAPLWHHVAPVAGQLHSVAFLTLALVLALACCTSNVTFLPFLSHLPPPFLRSFFLGQGLSALLPCVLALVQGVGRLECSPAPTNGTSGPPLNFPERFPASTFFWALTALLVTSAAAFQGLLLLLPSLPSVTTGGAGPELPLGSPGAEEEEKEEEEALPLQEPPSQAAGTIPGPDPEAHQLFSAHGAFLLGLLAITSALTNGVLPAVQSFSCLPYGRLAYHLAVVLGSAANPLACFLAMGVLCRSLAGLVGLSLLGMLFGAYLMVLAILSPCPPLVGTTAGVVLVVLSWVLCLCVFSYVKVAASSLLHGGGRPALLAXGVAIQVGSLLGAGTMFPPTSIYHVFQSRKDCV

SEQ ID NO: 32 - protein, 397 aa, artificial sequence
  Rat PAR-2
MRSLSLAWLLGGITLLAASASCNRTVNAPGPNSKGRSLIGRLDTPPPITGKGAPVEPGFSVDEFSASVLTGKLTTVFLPVIYIIVFVIGLPSNGMALWVFFFRTKKKHPAVIYMANLALADLLSVIWFPLKISYHLHGNDWTYGDALCKVLIGFFYGNMYCSILFMTCLSVQRYWVIVNPMGHSRKRANIAVGVSLAIWLLIFLVTIPLYVMRQTIYIPALNITTCHDVLPEEVLVGDMFSYFLSLAIGVFLFPALLTASAYVLMIKTLRSSAMDEHSEKKRRRAIRLIITVLSMYFICFAPSNVLLVVHYFLIKSQRQSHVYALYLVALCLSTLNSCIDPFVYYFVSKDFRDQARNALLCRSVRTVKRMQISLTSNKFSRKSSSYSSSSTSVKTSY

SEQ ID NO: 33 - protein, 327 aa, artificial sequence
  Human heavy chain IgG4 constant region
ASTKGPSVFPLAPCSRSTSESTAALGCLVKDYFPEPVTVSWNSGALTSGVHTFPAVLQSSGLYSLSSVVTVPSSSLGTKTYTCNVDHKPSNTKVDKRVESKYGPPCPSCPAPEFLGGPSVFLFPPKPKDTLMISRTPEVTCVVVDVSQEDPEVQFNWYVDGVEVHNAKTKPREEQFNSTYRVVSVLTVLHQDWLNGKEYKCKVSNKGLPSSIEKTISKAKGQPREPQVYTLPPSQEEMTKNQVSLTCLVKGFYPSDIAVEWESNGQPENNYKTTPPVLDSDGSFFLYSRLTVDKSRWQEGNVFSCSVMHEALHNHYTQKSLSLSLGK

SEQ ID NO: 34 - protein, 326 aa, artificial sequence
  human heavy chain IgG4 constant region (with S228P and terminal lysine deletion)
ASTKGPSVFPLAPCSRSTSESTAALGCLVKDYFPEPVTVSWNSGALTSGVHTFPAVLQSSGLYSLSSVVTVPSSSLGTKTYTCNVDHKPSNTKVDKRVESKYGPPCPPCPAPEFLGGPSVFLFPPKPKDTLMISRTPEVTCVVVDVSQEDPEVQFNWYVDGVEVHNAKTKPREEQFNSTYRVVSVLTVLHQDWLNGKEYKCKVSNKGLPSSIEKTISKAKGQPREPQVYTLPPSQEEMTKNQVSLTCLVKGFYPSDIAVEWESNGQPENNYKTTPPVLDSDGSFFLYSRLTVDKSRWQEGNVFSCSVMHEALHNHYTQKSLSLSLG

SEQ ID NO: 35 - protein, 330 aa, artificial sequence [sequence omitted]

SEQ ID NO: 36 - protein, 326 aa, artificial sequence
  Human heavy chain IgG2 constant region
ASTKGPSVFPLAPCSRSTSESTAALGCLVKDYFPEPVTVSWNSGALTSGVHTFPAVLQSSGLYSLSSVVTVPSSNFGTQTYTCNVDHKPSNTKVDKTVERKCCVECPPCPAPPVAGPSVFLFPPKPKDTLMISRTPEVTCVVVDVSHEDPEVQFNWYVDGVEVHNAKTKPREEQFNSTFRVVSVLTVVHQDWLNGKEYKCKVSNKGLPAPIEKTISKTKGQPREPQVYTLPPSREEMTKNQVSLTCLVKGFYPSDISVEWESNGQPENNYKTTPPMLDSDGSFFLYSKLTVDKSRWQQGNVFSCSVMHEALHNHYTQKSLSLSPGK

SEQ ID NO: 37 - protein, 107 aa, artificial sequence [sequence omitted]

SEQ ID NO: 38 - protein, 232 aa, artificial sequence
  IgG1 Fc domain
EPKSCDKTHTCPPCPAPELLGGPSVFLFPPKPKDTLMISRTPEVTCVVVDVSHEDPEVKFNWYVDGVEVHNAKTKPREEQYNSTYRVVSVLTVLHQDWLNGKEYKCKVSNKALPAPIEKTISKAKGQPREPQVYTLPPSRDELTKNQVSLTCLVKGFYPSDIAVEWESNGQPENNYKTTPPVLDSDGSFFLYSKLTVDKSRWQQGNVFSCSVMHEALHNHYTQKSLSLSPGK

SEQ ID NO: 39 - protein, 231 aa, artificial sequence
  Human IgG1 Fc domain (without C-terminal lysine residue)
EPKSCDKTHTCPPCPAPELLGGPSVFLFPPKPKDTLMISRTPEVTCVVVDVSHEDPEVKFNWYVDGVEVHNAKTKPREEQYNSTYRVVSVLTVLHQDWLNGKEYKCKVSNKALPAPIEKTISKAKGQPREPQVYTLPPSRDELTKNQVSLTCLVKGFYPSDIAVEWESNGQPENNYKTTPPVLDSDGSFFLYSKLTVDKSRWQQGNVFSCSVMHEALHNHYTQKSLSLSPG

SEQ ID NO: 40 - protein, 232 aa, artificial sequence
  IgG1 Fc
EPKSCDKTHTCPPCPAPELLGGPSVFLFPPKPKDTLMISRTPEVTCVVVDVSHEDPEVKFNWYVDGVEVHNAKTKPREEQYNSTYRVVSVLTVLHQDWLNGKEYKCKVSSKAFPAPIEKTISKAKGQPREPQVYTLPPSRDELTKNQVSLTCLVKGFYPSDIAVEWESNGQPENNYKTTPPVLDSDGSFFLYSKLTVDKSRWQQGNVFSCSVMHEALHNHYTQKSLSLSPGK

SEQ ID NO: 41 - protein, 232 aa, artificial sequence
  IgG1 Fc domain (with K322A)
EPKSCDKTHTCPPCPAPELLGGPSVFLFPPKPKDTLMISRTPEVTCVVVDVSHEDPEVKFNWYVDGVEVHNAKTKPREEQYNSTYRVVSVLTVLHQDWLNGKEYKCAVSNKALPAPIEKTISKAKGQPREPQVYTLPPSRDELTKNQVSLTCLVKGFYPSDIAVEWESNGQPENNYKTTPPVLDSDGSFFLYSKLTVDKSRWQQGNVFSCSVMHEALHNHYTQKSLSLSPGK

SEQ ID NO: 42 - protein, 229 aa, artificial sequence
  human IgG4 Fc
ESKYGPPCPSCPAPEFLGGPSVFLFPPKPKDTLMISRTPEVTCVVVDVSQEDPEVQFNWYVDGVEVHNAKTKPREEQFNSTYRVVSVLTVLHQDWLNGKEYKCKVSNKGLPSSIEKTISKAKGQPREPQVYTLPPSQEEMTKNQVSLTCLVKGFYPSDIAVEWESNGQPENNYKTTPPVLDSDGSFFLYSRLTVDKSRWQEGNVFSCSVMHEALHNHYTQKSLSLSLGK

SEQ ID NO: 43 - protein, 229 aa, artificial sequence
  human IgG4 Fc (with S228P)
ESKYGPPCPPCPAPEFLGGPSVFLFPPKPKDTLMISRTPEVTCVVVDVSQEDPEVQFNWYVDGVEVHNAKTKPREEQFNSTYRVVSVLTVLHQDWLNGKEYKCKVSNKGLPSSIEKTISKAKGQPREPQVYTLPPSQEEMTKNQVSLTCLVKGFYPSDIAVEWESNGQPENNYKTTPPVLDSDGSFFLYSRLTVDKSRWQEGNVFSCSVMHEALHNHYTQKSLSLSLGK

SEQ ID NO: 44 - protein, 228 aa, artificial sequence
  IgG4 Fc (with S228P and without terminal lysine residue)
ESKYGPPCPPCPAPEFLGGPSVFLFPPKPKDTLMISRTPEVTCVVVDVSQEDPEVQFNWYVDGVEVHNAKTKPREEQFNSTYRVVSVLTVLHQDWLNGKEYKCKVSNKGLPSSIEKTISKAKGQPREPQVYTLPPSQEEMTKNQVSLTCLVKGFYPSDIAVEWESNGQPENNYKTTPPVLDSDGSFFLYSRLTVDKSRWQEGNVFSCSVMHEALHNHYTQKSLSLSLG

SEQ ID NO: 45 - protein, 6 aa, artificial sequence
  PAR-2  activating ligand
SLIGKV

SEQ ID NO: 46 - protein, 6 aa, artificial sequence
  PAR-2
SLIGRL

SEQ ID NO: 47 - protein, 55 aa, artificial sequence
  human PAR-1
MGPRRLLLVAACFSLCGPLLSARTRARRPESKATNATLDPRSFLLRNPNDKYEPF

SEQ ID NO: 48 - protein, 398 aa, artificial sequence
  Nt-PAR-2
MRSPSAAWLLGAAILLAASLSCSGTIQGTNRSSKGRSLIGKVDGTSHVTGKGVTVETVFSVDEFSASVLTGKLTTLFVPSVYTGVFVVSLPLNIMAIVVFILKMKVKKPAVVYMLHLATADVLFVSVLPFKISYYFSGSDWQFGSELCRFVTAAFYCNMYASILLMTVISIDRFLAVVYPMQSLSWRTLGRASFTCLAIWALAIAGVVPLLLKEQTIQVPGLNITTCHDVLNETLLEGYYAYYFSAFSAVFFFVPLIISTVCYVSIIRCLSSSAVANRSKKSRALFLSAAVFCIFIICFGPTNVLLIAHYSFLSHTSTTEAAYFAYLLCVCVSSISCCIDPLIYYYASSECQRYVYSILCCKESSDPSSYNSSGQLMASKMDTCSSNLNNSIYKKLLT

SEQ ID NO: 49 - protein, 106 aa, artificial sequence
  Anti-PAR-2 antibody Ab1 light chain
QIVLSQSPAILSASPGEKVTMTCRASSSLPYIHWYQQKPGSSPRPWIYATSNLASGVPARFSGRGSGTSYSLTISRMEAEDAATYYCQQWSSTPPTFGGGSKLEIK

SEQ ID NO: 50 - protein, 121 aa, artificial sequence
  Anti-PAR-2 antibody Ab1 heavy chain
EVQLVEFGGGLVQPKGSLKLSCAASGFTFNTNAMHWVRQAPGKGLEWVARIGSKSSYFATYYADSVKDRFTISRDDSRSMFYLQMNNLKTEDTAMYYCVREDYYGSSFDLWGQGTTLTVSS

SEQ ID NO: 51 - protein, 111 aa, artificial sequence
  Anti-PAR-2 antibody Ab5 light chain
DIVLTQSPTSLAVSLGQRATISCRASESVDSYGNSFLHWYQQKAGQPPKLLIYRTSNLESGIPARFSGSGSRTDFTLTINPVEADDVATYFCQQSNEDPYTFGGGTKLELK

SEQ ID NO: 52 - protein, 123 aa, artificial sequence
  Anti-PAR-2 antibody Ab5 heavy chain
QVQLQQPGSELVKPGASVKLSCKASGYTFTNYWMHWVKQRPGQGLEWIGMIHPNSDFSNYNEKFKKKATLTVDKSSSTAYMQLSSLTSEDSAVYFCAKGPNYYGSRYWYFDVWGTGTTVTVSS

SEQ ID NO: 53 - protein, 106 aa, artificial sequence
  Anti-PAR-2 antibody Ab20 light chain
QIVLSQSPAILSASPGEKVTMTCRTSSSVIYIHWYQQKSGSSPKPWIYATSNLASGVPTRFSGSGSGTSYSLTISRVEAEDAATYYCHHWRSNPPTFGGGTKLEIK

SEQ ID NO: 54 - protein, 121 aa, artificial sequence
  Anti-PAR-2 antibody Ab20 heavy chain
EVQLVESGGGLVQPKGSLKLSCAASGFTFNIYAMHWVRQAPGKGLEWVARIGSKSSNYATNYADSVKDRFTISRDDSQSMLCLQMNNLKTEDTAMYYCVREDYYGNSFDSWGQGTTLAVSS

SEQ ID NO: 55 - protein, 106 aa, artificial sequence
  Anti-PAR-2 antibody Ab39 light chain
QIVLSQSPVILSTSPGEKVTMTCRANSRVIYVHWYQQKPGSSPKPWIFATSNLASGVPSRFSGSGSGTSYSLTISRVETEDAATYYCQHCGNNPPTFGSGTKLEIK

SEQ ID NO: 56 - protein, 121 aa, artificial sequence
  Anti-PAR-2 antibody Ab39 heavy chain
EVQLVESGGGLVQPKGSLKLSCAASGFTFNTYAMHWVRQAPGKGLEWVARIGSKSSYYATYYADSVKDRFTISRADSQSMLYLQMNNLKTEDTAIYYCVREDYYGCSFDYWGQGTTLTVSS

SEQ ID NO: 57 - protein, 107 aa, artificial sequence
  Anti-PAR-2 antibody Ab77 light chain
DIVMTQSHKFMSISVGDRVSITCKASQDVGTAVAWHQQKAGQSPKLLIYWASARHTGVPDRFTGSGSGTDFTLTISNVQSEDLTDFFCQQYSNYPFTFGSGTKLEIK

SEQ ID NO: 58 - protein, 121 aa, artificial sequence
  Anti-PAR-2 antibody Ab77 heavy chain
EVQLVGSGGGLVQPKGSLKLSCAASGFTFNTYAMHWVRQAPGKGLEWVARIGSKSSYYATYYADSVKDRFTISRDDSQSMLYLQMNNLKTEDTAMYYCVREDYYGSSYDYWGQGTTLTVSS

SEQ ID NO: 59 - protein, 107 aa, artificial sequence
  Anti-PAR-2 antibody Ab84 light chain
DIVMTQSHKFMSTSVGDRVSITCKASQDVGSAVAWHQQKPGQSPKLLIYWTSNRHTGVPDRFTGRRSGTDFTLTISNVQSEDLADYFCQQYSTYPFTFGSGTKLEIK

SEQ ID NO: 60 - protein, 121 aa, artificial sequence
  Anti-PAR-2 antibody Ab84 heavy chain
EVQLIESGGGLVQPKGSLKLSCAASGFTFNSYAMHWVRQAPGKGLEWVARIRSKNVHYATYYADSVKDRFTISRDDSQSMLYLQMNNLKTEDTAMYFCVREDYYGSSYDYWGQGTTLTVSS

SEQ ID NO: 61 - protein, 107 aa, artificial sequence
  Anti-PAR-2 antibody Ab86 light chain
DIVMTQSHKFMSTSLGDRVSITCKASQDVGSAVAWHQQKPGQSPKVLIYWASNRHTGVPDRFTGSGSGTDFTLTISNVQSEDLADYFCQQYSSYPFTFGSGTKLEIK

SEQ ID NO: 62 - protein, 121 aa, artificial sequence
  Anti-PAR-2 antibody Ab86 heavy chain
EVQLVESGGGLVQPKGSLKLSCAASGFTFNTYAMHWVRQAPGKGLEWVARIRSKNVHYATYYADSVKDRFTISRDDSQNMLYLQMNNLKTEDTAMYYCVREDYYGSSYDYWGQGTTLTVSS

SEQ ID NO: 63 - protein, 107 aa, artificial sequence
  Anti-PAR-2 antibody Ab87 light chain
DIVMTQSHKFMSTSVGDRVSITCKASQDVRSAVAWHQQKPGQSPKLLIYWASNRHTGVPDRFTGSGSGTDFTLTISNVQSEDLADYFCQQYSSYPFTFGSGTKLEIK

SEQ ID NO: 64 - protein, 121 aa, artificial sequence
  Anti-PAR-2 antibody Ab87 heavy chain
EVQLVESGGGLVQPKGSLKLSCAASGFTFYSYAMHWVRQAPGRGLEWVARIRSKNVHYATYYADSVKDRFTISRDDSQNMLYLQMNNLKTEDTAMYYCVREDYYGSSYDYWGQGTTLTVSS

SEQ ID NO: 65 - protein, 107 aa, artificial sequence
  Anti-PAR-2 antibody Ab114 light chain
DVQITQSPSYLAASPGETITINCRASKSISRYLAWYQEKPGKTNKLLIYSGSTLQSGVPSRFSGSGFGTDFTLTISSLEPEDFAMYYCQQHNKYPLTFGAGTKLELK

SEQ ID NO: 66 - protein, 123 aa, artificial sequence
  Anti-PAR-2 antibody Ab114 heavy chain
QVQLQQSGPELVKPGASVKISCKTSGFTFTSYYIHWVKQRPGQGLEWIGWIYPGSGNTYYNERFKGKATLTADTSSSTASMQLSSLTSEDSAVYYCANGPLFYGSSYWYFDVWGTGTTVTVSS

SEQ ID NO: 67 - protein, 108 aa, artificial sequence
  Anti-PAR-2 antibody Ab140 light chain
QIVLTQSPAIMSASLGERVTMTCTASSSVSSSYLHWYQQKPGSSPKLWIYATSNLASGVPARFSGSGSGTSYSLTISSMEAEDAATYYCHQYHRSPLTFGAGTKLELK

SEQ ID NO: 68 - protein, 121 aa, artificial sequence
  Anti-PAR-2 antibody Ab140 heavy chain
EVQLVESGGGLVQPKGSLKLSCAASGFTFNSYAMHWVRQAPGKGLEWVACIRSKSSYYATYYADSVKDRFTISRHDSQSMLYLQMNNLKTEDTAMYYCVREDYYGSSYDYWGQGTTLTVSS

SEQ ID NO: 69 - protein, 108 aa, artificial sequence
  Anti-PAR-2 antibody Ab189 light chain
QIVLTQSPAIMSASLGERVTMTCTASSSVISSYLHWYQQKPGSSPKLWIFSTSNLASGVPARFSGSGSGTSYSLTISTMEAEDAATYYCHQYHRSPLTFGAGTKLELK

SEQ ID NO: 70 - protein, 121 aa, artificial sequence
  Anti-PAR-2 antibody Ab189 heavy chain
EVQLVESGGGLVQPKGSLKLSCAASGFTFNTYAMHWVRQAPGKGLEWVARIRSKTTNYATYYADSVKDRFTISRDDSQSMLYLQISNLKTEDTAMYYCVREDYYGSSLDYWGQGTTLTVSS

SEQ ID NO: 71 - protein, 106 aa, artificial sequence
  Anti-PAR-2 antibody Ab192 light chain
ENVLTQSPAIMSASLGEKVTMSCRASSSVNYMYWYQQKSDASPKLWIYYTSNLAPGVPARFSGSGSGTSYSLTISSMEGEDAATYYCQQFTTSPYTFGGGTKLEIK

SEQ ID NO: 72 - protein, 121 aa, artificial sequence
  Anti-PAR-2 antibody Ab192 heavy chain
QVQLQQPGTELVKPGASVKLSCKASGYTFTSYWMHWIKQRPGQGLEWIGNINPSSGGTNYNEKFKTKATLTVDKSSSTAYMQLSSLTSEDSAVYYCAGEAYSNYVAWFAYWGQGTLVTVSS

SEQ ID NO: 73 - protein, 107 aa, artificial sequence
  Anti-PAR-2 antibody Ab201 light chain
EVQITQSPSYLAASPGETITINCRASKSISKYLAWYQEKPGKTNKLLIYSGSTLQSGIPSRFSGSGSGTDFTLTISSLEPEDFAMYYCQQHNKYPLTFGAGTRLELK

SEQ ID NO: 74 - protein, 123 aa, artificial sequence
  Anti-PAR-2 antibody Ab201 heavy chain
QVQLQQSGPELVKPGASVKISCKASGFSFTSFYIHWVNQRPGQGLEWIGWIYPGSGNTLYNEKFKGKATLTADTSSSTAYIHLSSLTSEDSAVYYCTRGPLFYGSSHWYFDVWGMGTTVTVSS

SEQ ID NO: 75 - protein, 106 aa, artificial sequence
  Anti-PAR-2 antibody Ab209 light chain
ENVLTQSPAIMSASLGEKVTMSCRASSSVNYMYWYRQKSDASPKLWIYYTSNLAPGVPTRFSGSGSGTSYSLTISSMEGEDAATYYCQQFTTSPYTFGGGTKLEIK

SEQ ID NO: 76 - protein, 121 aa, artificial sequence
  Anti-PAR-2 antibody Ab209 heavy chain
QVQLQQPGTELVKPGASVKLSCKASGYTFTSYWMHWIKQRPGQGLEWIGNINPSTGSTNFNVKFKTKATLTVDKSSSTTYMQLNSLTSEDSAVYYCAGEAYSNYVAWFAYWGQGTLVTVSS

SEQ ID NO: 77 - protein, 106 aa, artificial sequence
  Anti-PAR-2 antibody Ab225 light chain
EIVLTQSPTTMAASPGEKVTITCRASSSVRSMYWYQQKSGASPKPWIYETSKLTSGVPDRFSGSGSGTSYSFTISSMGTEDAGTYYCHQWTTTPYTFGAGTKLELK

SEQ ID NO: 78 - protein, 118 aa, artificial sequence
  Anti-PAR-2 antibody Ab225 heavy chain
QVQLKESGPGLVQPSQTLSLTCTVSGFSLTSYHVSWVRQSPGKGLEWMGIIWTGGSTAYNSLLKSRLSISRDTSKSQVFLKMNSLQTEDTATYYCARRGAYPFYFDYWGQGVMVTVSS

SEQ ID NO: 79 - protein, 107 aa, artificial sequence
  Anti-PAR-2 antibody Ab227 light chain
DIQMTQSPHSLSASLGETVSIECLASEGISNYLAWFQQKPGKSPQLLIYYASSLQDGVPSRFSGSGSGTQYSLKISNMQPEDEGVYYCQQGYKYPWTFGGGTELELK

SEQ ID NO: 80 - protein, 121 aa, artificial sequence
  Anti-PAR-2 antibody Ab227 heavy chain
EVQLVESGGGLVQPGRSLKLSCVASGFTFNNYWMTWIRQAPGKGLEWVASITNSGGRTYYPDSVKGRFTVSRDSAKSTLYLQMNSLRSEDTATYYCTRDRIIRGSTWFTYWGQGTLVTVSS

SEQ ID NO: 81 - protein, 107 aa, artificial sequence
  Anti-PAR-2 antibody Ab228 light chain
DIQMTQSPHSLSASLGETVSIECLASEGISNYLAWYQQKPGKSPQLLIYYASSLQDGVPSRFSGSGSGTQYSLKISNMQPEDEGVYYCHQGYKYPWTFGGGTKLELK

SEQ ID NO: 82 - protein, 121 aa, artificial sequence
  Anti-PAR-2 antibody Ab228 heavy  chain
EVQLVESGGGLVQPGRSLKLSCVVSGFTFNNYWMTWIRQAPGKGLEWVASITNSGGNTYYPDSVKGRFTISRDNAKSTLYLQMNSLRSEDTATYYCTRDRIIRGSTWFAYWGQGTLVTVSS

SEQ ID NO: 83 - protein, 106 aa, artificial sequence
  Anti-PAR-2 antibody Ab234 light chain
EIVLTQSPTTMAASPGEKVTLTCRASSSVIYMHWYQQRSGASPKLWIYETSKLASGVPNRFGGSGSGTSYSLTINSMETEDAATYYCQQGSYYPWTFGGGTKLELK

SEQ ID NO: 84 - protein, 120 aa, artificial sequence
  Anti-PAR-2 antibody Ab234 heavy chain
EVQLVETGGGLVQPGRSLKLSCVASGFTFNNYWLYWIRQAPGKGLEWVSSINNDGGGTYYPDSVKGRFTVSRDNAENTVYLQMNSLRSEDTATYYCARDRAFIRGRFAYWGQGTLVTVSS

SEQ ID NO: 85 - protein, 106 aa, artificial sequence
  Anti-PAR-2 antibody Ab245 light chain
EVVLTQSPTTMAASPGEKVTITCRATSSVSHMYWYQQKSGASPKPWIYETSKLASGVPDRFRGSGSGTSYSFTISSMETEDVATYYCHQWSSFPYTFGPGTKLELK

SEQ ID NO: 86 - protein, 118 aa, artificial sequence
  Anti-PAR-2 antibody Ab245 heavy chain
QVQLKESGPGLVQPSQTLFLTCTVSGFSLTSYHVSWVRQPPGKGLEWMGIIWTGGSTAYNSLLKPRLTISRDTSKSQVFLKMNSLRTEDTATYYCARRGLYPFYFDYWGQGVMVTVSS

SEQ ID NO: 87 - protein, 106 aa, artificial sequence
  Anti-PAR-2 antibody Ab248 light chain
EIVLTQSPTTLAASPGEKVTITCRASSRVSNMYWYQQKSGASPKAWIYETSKLASGVPDRFSGSGSGTSYSFTISSMETEDAATYYCHQWTSTPYTFGAGTKLELK

SEQ ID NO: 88 - protein, 118 aa, artificial sequence
  Anti-PAR-2 antibody Ab248 heavy chain
QVQLKESGPGLVQPSQTLSLTCTVSGFSLTNYHVSWVRQPPGKGLEWMGIIWTGGSTAYNSLLKSRLSISRDTSKSQVFLKMNSLQTEDTATYYCARRGLYPYYFDYWGQGVMVTVSS

SEQ ID NO: 89 - protein, 107 aa, artificial sequence
  Anti-PAR-2 antibody Ab261 light chain
DIQMTQSPHSLSASLGETVSIECLASEGISNYLAWFQQKPGKSPQLLIYYASSLQDGVPSRFSGSGSGTQYSLKISNMQPEDEGVYYCQQGYKYPWTFGGGTKLELK

SEQ ID NO: 90 - protein, 121 aa, artificial sequence
  Anti-PAR-2 antibody Ab261 heavy chain
EVQLVESGGGLVQPGRSLKLSCVASGFTFNNYWMTWIRQAPGKGLEWVASITNTGGNTYYPDSVKGRFTISRDNAKSTLYLQMNSLRSEDTATYYCTRDRIIRGADWFAYWGQGTLVTVSS

SEQ ID NO: 91 - protein, 106 aa, artificial sequence
  Anti-PAR-2 antibody Ab303 light chain
DIQMTQSPSFLSASVGERVTLSCKTSQKINRYLDWYQQKLGEAPKLLIYNTNNLHTGIPSRFSGSGSGTDYTLTISSLQPEDVATYFCLQHSSWPTFGAGTKLELK

SEQ ID NO: 92 - protein, 120 aa, artificial sequence
  Anti-PAR-2 antibody Ab303 heavy chain
QVTLKESGPGILQPSHTLSLTCSFSGFSLSTYGMGVSWIRQPSGKGLEWLASIWWNGNTYNNPSLKSRLTVSKDTSNNQAFLKVTSVDTADTATYYCAHTPNLGNWFAYWGQGTLVTVSS

SEQ ID NO: 93 - protein, 106 aa, artificial sequence
  Anti-PAR-2 antibody Ab311 light chain
DIQMTQSPSFLSASVGDRVTINCKASQNIYKYLDWYQQKLGEAPKLLIYNSNILHTGVPSRFSGSGSGTDFTLSISSLQPEDVATYFCLQHNSGWTFGGGSKLELR

SEQ ID NO: 94 - protein, 119 aa, artificial sequence
  Anti-PAR-2 antibody Ab311 heavy chain
QVQLKESGPGLVQPSQTLSLSCTVSGFSLTTYGVIWVRQPPGKGLMWMGVIWGNGNTYYNSPLKSRLSISRDTSKSQVFLKMNNLQSEDTAMYFCGRWRGYKDYPFDYWGQGVKVTVSS

SEQ ID NO: 95 - protein, 106 aa, artificial sequence
  Anti-PAR-2 antibody Ab313 light chain
DIQMTQSPSVLSASVGDRVILNCKASQKINKYLNWYQQKLGEAPKLLIYTTNNLQTGIPSRFSGSGSGTDFTLTISSLQPEDFATYFCFQHSSWPTFGAGTKLELK

SEQ ID NO: 96 - protein, 118 aa, artificial sequence
  Anti-PAR-2 antibody Ab313 heavy chain
EVQLKESGPGLVQPSQTLSLTCTVSGFSLTDYSVHWVRQPPGKGLEWMGVMWSGGSTSYNSPLKSRLSISRDTSKSQVFLKTNSLQTEDTAIYYCTRARPTVATLDYWGQGVMVTVSS

SEQ ID NO: 97 - protein, 106 aa, artificial sequence
  Anti-PAR-2 antibody Ab323 light chain
DIQMTQSPSFLSASVGDRVTINCKASQNIYKYLDWYQQKLGEAPKLLMYNTNTLHTGIPSRFSGSGSGTDFTLTISSLQPEDVATYFCLQHNSGWTFGGGTKLELK

SEQ ID NO: 98 - protein, 119 aa, artificial sequence
  Anti-PAR-2 antibody Ab323 heavy chain
QVQLKESGPGLVQPSQTLSLTCSVSGFSLSTYGIIWVRQPPGKGLEWMGVIWGNGNTHYNSALKSRLSITRDTSKSQVFLKMNNLQTEDTAMYFCGRWRGYKDYPFDYWGQGVMVTVSS

SEQ ID NO: 99 - protein, 106 aa, artificial sequence
  Anti-PAR-2 antibody Ab335 light chain
DIQMTQSPSFLSASVGDRVTINCKASRNIYKYLDWYQQKLGEAPKLLIYNTNNLHTGIPSRFSGSGSGTDFTLTISSLQPEDVATYFCLQHNSGWTFGGGTKLELK

SEQ ID NO: 100 - protein, 119 aa, artificial sequence
  Anti-PAR-2 antibody Ab335 heavy chain
QVQLKESGPGLVQPSQTLSLSCTVSGFSLSTYGVIWVRQPPGKGLEWMGVIWGNGNTNYNSALKSRLSISRDTSKSQVFLKMNNLQSEDTAMYFCGRWRGYKDYPFDYWGQGVKVTVSS

SEQ ID NO: 101 - protein, 106 aa, artificial sequence
  Anti-PAR-2 antibody Ab342 light chain
DIQMTQTPSFLSASVGDRVTINCRASQNIYKYLDWYQLKLGEAPKLLIYNTNTLHTGIPSRFSGSGSGTDFTLTISSLQPEDVATYFCLQHNSGWAFGGGTKLELK

SEQ ID NO: 102 - protein, 119 aa, artificial sequence
  Anti-PAR-2 antibody Ab342 heavy chain
QVQLKESGPGLVQPSQTLSLSCTVSGFSLNTYGVIWVRQPPGKGLDWMGVIWGNGNTYYDSALKSRLSISRDTSKSQIFLKMNNLQSEDTAMYFCGRWRGFKDYPFDYWGQGVKVTVSS

SEQ ID NO: 103 - protein, 107 aa, artificial sequence
  Anti-PAR-2 antibody Ab343 light chain
DIQMTQSPHSLSASLGETVSIECLASEAISNYLAWYQQKPGKSPQLLIYYASSLKDGVPSRISGSGSGTQYSLKISNMQPEDEGVYYCQQGYKYPRTFGGGTKLELK

SEQ ID NO: 104 - protein, 121 aa, artificial sequence
  Anti-PAR-2 antibody Ab343 heavy chain
EVQLVESGGGLVQPGRSLKLSCVASGFTFNNYWMSWIRQAPGKGLEWVASITNTGGRIFYPDSVKGRFTISRDNAQNTLYLQMNSLRSEDAATYYCTRDRLYYGSNWFTYWGQGTLVTVSS

SEQ ID NO: 105 - protein, 106 aa, artificial sequence
  Anti-PAR-2 antibody Ab348 light chain
DIQMTQSPSFLSASVGDRVTINCKASQNIYKYLDWYQQKLGEAPKLLIYNTNSLHTGIPSRFSGSGSGTDFTLTISSLQPEDVATYFCLQHNSGWTFGGGTKLELK

SEQ ID NO: 106 - protein, 119 aa, artificial sequence
  Anti-PAR-2 antibody Ab348 heavy chain
QVQLKESGPGLVQPSQTLSLTCSVSGFSLSSYGVIWVRQPPGKGLEWMGVVWGNGNTAYNFTLKSRLTISRDTSKSQVFLKMNNLQTEDTAMYFCGRWRGFKDYPFDYWGQGVMVTVSS

SEQ ID NO: 107 - protein, 105 aa, artificial sequence
  Anti-PAR-2 antibody Ab360 light chain
DTVLTQSPALAVSPGERVTISCRASESVRTRMHWYQQRPGQQPKLLIYGASNPESGVPARFSGSGSGTDFTLTIDPVEADDSATYFCHQSWNEYTFGAGTKLELK

SEQ ID NO: 108 - protein, 120 aa, artificial sequence
  Anti-PAR-2 antibody Ab360 heavy chain
EVQLVESGGGLVQPGRSLKLSCVASGFTFNNYWMTWIRQAPGKGLEWVASITNTGGSTYYPDSVKGRFTISRDNAKSTLYLQMNSLRSEDTATYYCTREGIRGTGWFAYWGQGTLVTVSS

SEQ ID NO: 109 - protein, 372 aa, artificial sequence
  human PAR-2 (without the signal sequence)
IQGTNRSSKGRSLIGKVDGTSHVTGKGVTVETVFSVDEFSASVLTGKLTTVFLPIVYTIVFVVGLPSNGMALWVFLFRTKKKHPAVIYMANLALADLLSVIWFPLKIAYHIHGNNWIYGEALCNVLIGFFYGNMYCSILFMTCLSVQRYWVIVNPMGHSRKKANIAIGISLAIWLLILLVTIPLYVVKQTIFIPALNITTCHDVLPEQLLVGDMFNYFLSLAIGVFLFPAFLTASAYVLMIRMLRSSAMDENSEKKRKRAIKLIVTVLAMYLICFTPSNLLLVVHYFLIKSQGQSHVYALYIVALCLSTLNSCIDPFVYYFVSHDFRDHAKNALLCRSVRTVKQMQVSLTSKKHSRKSSSYSSSSTTVKTSY

SEQ ID NO: 110 - protein, 107 aa, artificial sequence; identical to SEQ ID NO: 89
  Anti-PAR-2 antibody Ab380 light chain

SEQ ID NO: 111 - protein, 121 aa, artificial sequence
  Anti-PAR-2 antibody Ab380 heavy  chain
EVQLVESGGGLVQPGRSLKLSCVATGFTFNNYWMTWIRQAPGKGLEWVASITNSGGNTYYPDSVKGRFTISRDDAKSTLYLQMNSLRSEDTATYYCTRVRVYYGSNWFVYWGQGTLVTVSS

SEQ ID NO: 112 - protein, 107 aa, artificial sequence
  Anti-PAR-2 antibody Ab392 light chain
DIQMTQSPHSLSASLGEGVSIECLASEGISNYLAWFQQKPGKSPQLLIYYASSLQDGVPSRFSGSGSGTQYSLKISNMQPEDEGVYYCQQGYKYPWTFGGGTKLELK

SEQ ID NO: 113 - protein, 121 aa, artificial sequence
  Anti-PAR-2 antibody Ab392 heavy chain
EVQLVESGGGLVQPGRSLKLSCVASGFTFNNKWMTWIRQAPGKGLEWIASITNTGGRTFYPDSVKGRFTISRDDAKSTLYLQMNSLRSEDTATYYCTRATIRRGASYFDYWGQGVMVTVSS

SEQ ID NO: 114 - protein, 107 aa, artificial sequence
  Anti-PAR-2 antibody Ab435 light chain
DIQMTQSPHSLSASLGETVSIECLASEGISNYLAWYQQKPGKSPQLLIYYASSLQDGVPSRFSGSGSGTQYSLKISNMQPEDEGIYYCQQHYKYPWTFGGGTKLELK

SEQ ID NO: 115 - protein, 121 aa, artificial sequence
  Anti-PAR-2 antibody Ab435 heavy chain
EVQLVESGGGLVQPGRSLKLSCVGSGFTFNNYWMTWIRQAPGWGLEWVASITNTGGRTYYPDSVKGRFTISRDNAKSTLYLQMNSLRSEDTATYYCTRDRVYYGSNWFVYWGQGTLVTVSS

SEQ ID NO: 116 - protein, 119 aa, artificial sequence
  Anti-PAR-2 antibody (309) Variable heavy CHain Sequence
QVQLKESGPGLVQPSQTLSLTCTVSGFSLNSYGVIWARQPPGKGLDWMGVIWGNGNTYYNSDLKSRLSISRDTSKSQVFLKMNNLQAEDTALYFCARWRGYKDYPFDYWGQGVMVTVSS

SEQ ID NO: 117 - protein, 106 aa, artificial sequence
  Anti-PAR-2 antibody (309) Variable Light CHain Sequence
DIQMTQSPSFLSASVGDRVTFNCKASQNIYKYLDWYQQKLGEAPKLLIYNTNSLHTGIPSRFSGSGFGTDFTLTISSLQPEDVATYFCLQHNSGWTFGGGTKLELR

SEQ ID NO: 118 - protein, 119 aa, artificial sequence
  Anti-PAR-2 antibody (309-6e and 309-6i) Variable Heavy Chain Sequence
EVQLVESGGGLVQPGGSLRLSCAASGFSLNSYGVIWVRQAPGKGLEWVSVIWGNGNTYYNDSVKGRFTISRDNSKNTLYLQMNSLRAEDTAVYYCARWRGYKDYPFDYWGQGTLVTVSS

SEQ ID NO: 119 - protein, 119 aa, artificial sequence
  Anti-PAR-2 antibody (309-11e and 309-11i) Variable Heavy Chain Sequence
QVQLQESGPGLVKPSETLSLTCTVSGFSLNSYGVIWIRQPPGKGLEWIGVIWGNGNTYYNPSLKSRVTISVDTSKNQFSLKLSSVTAADTAVYYCARWRGYKDYPFDYWGQGTLVTVSS

SEQ ID NO: 120 - protein, 119 aa, artificial sequence
  Anti-PAR-2 antibody (309-12e and 309-12i) Variable Heavy Chain Sequence
QVQLQQWGAGLLKPSETLSLTCAVYGFSLNSYGVIWIRQPPGKGLEWIGVIWGNGNTYYNPSLKSRVTISVDTSKNQFSLKLSSVTAADTAVYYCARWRGYKDYPFDYWGQGTLVTVSS

SEQ ID NO: 121 - protein, 106 aa, artificial sequence
  Anti-PAR-2 antibody (309-4i, 309-6i,309-11i, and 309-12i) Variable Light Chain Sequence
DIQMTQSPSSLSASVGDRVTITCKASQNIYKYLDWYQQKPGKAPKRLIYNTNSLHTGVPSRFSGSGSGTEFTLTISSLQPEDFATYYCLQHNSGWTFGGGTKVEIK

SEQ ID NO: 122 - protein, 119 aa, artificial sequence
  Anti-PAR-2 antibody P24E5 Variable Heavy Chain Sequence
QVQLVQSGAEVKKPGSSVKVSCKASGFSLSSYGVIWVRQAPGQGLEWMGVIWGNGNTYYNQKFQGRVTITADESTSTAYMELSSLRSEDTAVYYCARWRGYKDYPFDYWGQGTLVTVSS

SEQ ID NO: 123 - protein, 119 aa, artificial sequence; identical to SEQ ID NO: 122
  Anti-PAR-2 antibody P24E9 Variable Heavy Chain Sequence

SEQ ID NO: 124 - protein, 119 aa, artificial sequence
  Anti-PAR-2 antibody P24E22 Variable Heavy Chain Sequence
QVQLVQSGAEVKKPGSSVKVSCKASGFSLNSYGVIWVRQAPGQGLEWMGVIWGNGNTYYAQKFQGRVTITADESTSTAYMELSSLRSEDTAVYYCARWRGYKDYPFDYWGQGTLVTVSS

SEQ ID NO: 125 - protein, 106 aa, artificial sequence
  Anti-PAR-2 antibody P24E27 VAriable Light Chain Sequence
EIVLTQSPATLSLSPGERATLSCRASQNIYKYLDWYQQKPGQAPRLLIYNTNSLHTGIPARFSGSGSGRDFTLTISSLEPEDFAVYYCLQHNSGWTFGGGTKVEIK

SEQ ID NO: 126 - protein, 106 aa, artificial sequence
  Anti-PAR-2 antibody P24E29 VAriable Light Chain Sequence
EIVLTQSPATLSLSPGERATLSCKASQNVYKYLDWYQQKPGQAPRLLIYNTNSLHTGIPARFSGSGSGRDFTLTISSLEPEDFAVYYCLQHNSGWTFGGGTKVEIK

SEQ ID NO: 127 - protein, 106 aa, artificial sequence
  Anti-PAR-2 antibody P24E36 VAriable Light Chain Sequence
EIVLTQSPATLSLSPGERATLSCKASQNIYKYLDWYQQKPGQAPRLLIYNANSLHTGIPARFSGSGSGRDFTLTISSLEPEDFAVYYCLQHNSGWTFGGGTKVEIK

SEQ ID NO: 128 - protein, 106 aa, artificial sequence
  Anti-PAR-2 antibody P24E39 VAriable Light Chain Sequence
EIVLTQSPATLSLSPGERATLSCKASQNIYKYLDWYQQKPGQAPRLLIYNTNSRHTGIPARFSGSGSGRDFTLTISSLEPEDFAVYYCLQHNSGWTFGGGTKVEIK

SEQ ID NO: 129 - protein, 106 aa, artificial sequence
  Anti-PAR-2 antibody P24E40 VAriable Light Chain Sequence
EIVLTQSPATLSLSPGERATLSCKASQNIYKYLDWYQQKPGQAPRLLIYNTNSLATGIPARFSGSGSGRDFTLTISSLEPEDFAVYYCLQHNSGWTFGGGTKVEIK

SEQ ID NO: 130 - protein, 106 aa, artificial sequence
  Anti-PAR-2 antibody P24E41 VAriable Light Chain Sequence
EIVLTQSPATLSLSPGERATLSCKASQNIYKYLDWYQQKPGQAPRLLIYDASNRATGIPARFSGSGSGRDFTLTISSLEPEDFAVYYCLQHNSGWTFGGGTKVEIK

SEQ ID NO: 131 - protein, 106 aa, artificial sequence
  Anti-PAR-2 antibody P24E60 VAriable Light Chain Sequence
EIVLTQSPATLSLSPGERATLSCKASQNIYKWLDWYQQKPGQAPRLLIYNTNSLHTGIPARFSGSGSGRDFTLTISSLEPEDFAVYYCLQHNSGWTFGGGTKVEIK

SEQ ID NO: 132 - protein, 106 aa, artificial sequence
  Anti-PAR-2 antibody P24E61 VAriable Light Chain Sequence
EIVLTQSPATLSLSPGERATLSCKASQNIYKFLDWYQQKPGQAPRLLIYNTNSLHTGIPARFSGSGSGRDFTLTISSLEPEDFAVYYCLQHNSGWTFGGGTKVEIK

SEQ ID NO: 133 - protein, 119 aa, artificial sequence
  Anti-PAR-2 antibody P24E186 VAriable Heavy Chain Sequence
QVQLVQSGAEVKKPGSSVKVSCKASGFSLNSYGVIWVRQAPGQGLEWMGVIWGNGNTYYNQKFQGRVTITADESTSTAYMELSSLRSEDTAVYYCARWRGWKDYPFDYWGQGTLVTVSS

SEQ ID NO: 134 - protein, 119 aa, artificial sequence
  Anti-PAR-2 antibody P24E216 VAriable Heavy Chain Sequence
QVQLVQSGAEVKKPGSSVKVSCKASGFSLNYYGVIWVRQAPGQGLEWMGVIWGNGNTYYNQKFQGRVTITADESTSTAYMELSSLRSEDTAVYYCARWRGYKDYPFDYWGQGTLVTVSS

SEQ ID NO: 135 - protein, 119 aa, artificial sequence
  Anti-PAR-2 antibody P24E219 VAriable Heavy Chain Sequence
QVQLVQSGAEVKKPGSSVKVSCKASGFSLNSYGGIWVRQAPGQGLEWMGVIWGNGNTYYNQKFQGRVTITADESTSTAYMELSSLRSEDTAVYYCARWRGYKDYPFDYWGQGTLVTVSS

SEQ ID NO: 136 - protein, 119 aa, artificial sequence
  Anti-PAR-2 antibody P24E232 VAriable Heavy Chain Sequence
QVQLVQSGAEVKKPGSSVKVSCKASGFSLNSYGVIWVRQAPGQGLEWMGVIWGNGNTYYGQKFQGRVTITADESTSTAYMELSSLRSEDTAVYYCARWRGYKDYPFDYWGQGTLVTVSS

SEQ ID NO: 137 - protein, 119 aa, artificial sequence
  Anti-PAR-2 antibody P24E233 VAriable Heavy Chain Sequence
QVQLVQSGAEVKKPGSSVKVSCKASGFSLNSYGVIWVRQAPGQGLEWMGVIWGNGNTYYYQKFQGRVTITADESTSTAYMELSSLRSEDTAVYYCARWRGYKDYPFDYWGQGTLVTVSS

SEQ ID NO: 138 - protein, 119 aa, artificial sequence
  Anti-PAR-2 antibody (P24E278,P24E279,P24E280,P24E280,andP24E282) VAriable Heavy Chain Sequence
QVQLVQSGAEVKKPGSSVKVSCKASGFSLSSYGVIWVRQAPGQGLEWMGVIWGNGNTYYAQKFQGRVTITADESTSTAYMELSSLRSEDTAVYYCARWRGYKDYPFDYWGQGTLVTVSS

SEQ ID NO: 139 - protein, 119 aa, artificial sequence
  Anti-PAR-2 antibody (P24E283,P24E284,P24E285,P24E286,and P24E287) VAriable Heavy Chain Sequence
QVQLVQSGAEVKKPGSSVKVSCKASGFSLNSYAVIWVRQAPGQGLEWMGVIWGNGNTYYAQKFQGRVTITADESTSTAYMELSSLRSEDTAVYYCARWRGYKDYPFDYWGQGTLVTVSS

SEQ ID NO: 140 - protein, 119 aa, artificial sequence
  Anti-PAR-2 antibody (P24E288,P24E289,P24E290,P24E291,and P24E292) VAriable Heavy Chain Sequence
QVQLVQSGAEVKKPGSSVKVSCKASGFSLNSYGIIWVRQAPGQGLEWMGVIWGNGNTYYAQKFQGRVTITADESTSTAYMELSSLRSEDTAVYYCARWRGYKDYPFDYWGQGTLVTVSS

SEQ ID NO: 141 - protein, 119 aa, artificial sequence
  Anti-PAR-2 antibody (P24E293,P24E294,P24E295,P24E296,and P24E297) VAriable Heavy Chain Sequence
QVQLVQSGAEVKKPGSSVKVSCKASGFSLNSYAISWVRQAPGQGLEWMGVIWGNGNTYYAQKFQGRVTITADESTSTAYMELSSLRSEDTAVYYCARWRGYKDYPFDYWGQGTLVTVSS

SEQ ID NO: 142 - protein, 119 aa, artificial sequence
  Anti-PAR-2 antibody (P24E298,P24E743,P24E794,P24E833,and P24E889) VAriable Heavy Chain Sequence
QVQLVQSGAEVKKPGSSVKVSCKASGFSLSSYAISWVRQAPGQGLEWMGVIWGNGNTYYAQKFQGRVTITADESTSTAYMELSSLRSEDTAVYYCARWRGYKDYPFDYWGQGTLVTVSS

SEQ ID NO: 143 - protein, 119 aa, artificial sequence
  Anti-PAR-2 antibody (P24E300,P24E922,P24E923,and P24E924) VAriable Heavy Chain Sequence
QVQLVQSGAEVKKPGSSVKVSCKASGFSLSSYAISWVRQAPGQGLEWMGVIWGNGNTYYAQKFQGRVTITADESTSTAYMELSSLRSEDTAVYYCARWRGWKDYPFDYWGQGTLVTVSS

SEQ ID NO: 144 - protein, 119 aa, artificial sequence
  Anti-PAR-2 antibody (P24E301,P24E914,P24E915,P24E916,P24E917,and P24E933) VAriable Heavy Chain Sequence
QVQLVQSGAEVKKPGSSVKVSCKASGFSLSSYAISWVRQAPGQGLEWMGVIWGNGNTYYAQKFQGRVTITADESTSTAYMELSSLRSEDTAVYYCARWKGYKDYPFDYWGQGTLVTVSS

SEQ ID NO: 145 - protein, 119 aa, artificial sequence
  Anti-PAR-2 antibody (P24E918,P24E919,P24E920,and P24E921) VAriable Heavy Chain Sequence
QVQLVQSGAEVKKPGSSVKVSCKASGFSLSSYAISWVRQAPGQGLEWMGVIWGNGNTYYAQKFQGRVTITADESTSTAYMELSSLRSEDTAVYYCARWRGFKDYPFDYWGQGTLVTVSS

SEQ ID NO: 146 - protein, 119 aa, artificial sequence
  Anti-PAR-2 antibody (P24E930,P24E931,P24E932,P24E971,P24E972,and P24E973) VAriable Heavy Chain Sequence
QVQLVQSGAEVKKPGSSVKVSCKASGFSLSSYAISWVRQAPGQGLEWMGVIWGNGNVYYAQKFQGRVTITADESTSTAYMELSSLRSEDTAVYYCARWKGYKDYPFDYWGQGTLVTVSS

SEQ ID NO: 147 - protein, 119 aa, artificial sequence
  Anti-PAR-2 antibody (P24E934,P24E935,and P24E936) VAriable Heavy Chain Sequence
QVQLVQSGAEVKKPGSSVKVSCKASGFSLSSYAISWVRQAPGQGLEWMGVIWGNGNVYYAQKFQGRVTITADESTSTAYMELSSLRSEDTAVYYCARWKGYKDHPFDYWGQGTLVTVSS

SEQ ID NO: 148 - protein, 106 aa, artificial sequence
  Anti-PAR-2 antibody (P24E936 and P24E973) Variable Light Chain Sequence
EIVLTQSPATLSLSPGERATLSCRASQNVYKWLDWYQQKPGQAPRLLIYNAYSRATGIPARFSGSGSGRDFTLTISSLEPEDFAVYYCQQHGHGWTFGGGTKVEIK

SEQ ID NO: 149 - protein, 106 aa, artificial sequence
  Anti-PAR-2 antibody (P24E279,P24E284,P24E289,and P24E294) Variable Light Chain Sequence
EIVLTQSPATLSLSPGERATLSCRASQNIYKYLDWYQQKPGQAPRLLIYNTNSLATGIPARFSGSGSGRDFTLTISSLEPEDFAVYYCLQHNSGWTFGGGTKVEIK

SEQ ID NO: 150 - protein, 106 aa, artificial sequence
  Anti-PAR-2 antibody (P24E280,P24E285,P24E290,and P24E295) Variable Light Chain Sequence
EIVLTQSPATLSLSPGERATLSCKASQNVYKYLDWYQQKPGQAPRLLIYNTNSLATGIPARFSGSGSGRDFTLTISSLEPEDFAVYYCLQHNSGWTFGGGTKVEIK

SEQ ID NO: 151 - protein, 106 aa, artificial sequence
  Anti-PAR-2 antibody (P24E281,P24E286,P24E291,and P24E296) Variable Light Chain Sequence
EIVLTQSPATLSLSPGERATLSCKASQNIYKYLDWYQQKPGQAPRLLIYNANSLATGIPARFSGSGSGRDFTLTISSLEPEDFAVYYCLQHNSGWTFGGGTKVEIK

SEQ ID NO: 152 - protein, 106 aa, artificial sequence
  Anti-PAR-2 antibody (P24E282,P24E287,P24E292,and P24E297) Variable Light Chain Sequence
EIVLTQSPATLSLSPGERATLSCKASQNIYKYLDWYQQKPGQAPRLLIYNTNSRATGIPARFSGSGSGRDFTLTISSLEPEDFAVYYCLQHNSGWTFGGGTKVEIK

SEQ ID NO: 153 - protein, 106 aa, artificial sequence
  Anti-PAR-2 antibody (P24E298,P24E300,and P24E301) Variable Light Chain Sequence
EIVLTQSPATLSLSPGERATLSCKASQNIYKWLDWYQQKPGQAPRLLIYNTNSLATGIPARFSGSGSGRDFTLTISSLEPEDFAVYYCLQHNSGWTFGGGTKVEIK

SEQ ID NO: 154 - protein, 106 aa, artificial sequence
  Anti-PAR-2 antibody (P24E743,P24E917,P24E921,and P24E931) Variable Light Chain Sequence
EIVLTQSPATLSLSPGERATLSCKASQNVYKWLDWYQQKPGQAPRLLIYNAYSLATGIPARFSGSGSGRDFTLTISSLEPEDFAVYYCQQHGSGWTFGGGTKVEIK

SEQ ID NO: 155 - protein, 106 aa, artificial sequence
  Anti-PAR-2 antibody (P24E794,P24E916,P24E920,and P24E924) Variable Light Chain Sequence
EIVLTQSPATLSLSPGERATLSCRASQNVYKWLDWYQQKPGQAPRLLIYNAYSRATGIPARFSGSGSGRDFTLTISSLEPEDFAVYYCQQHNSGWTFGGGTKVEIK

SEQ ID NO: 156 - protein, 106 aa, artificial sequence
  Anti-PAR-2 antibody (P24E883,P24E915,P24E919,and P24E923) Variable Light Chain Sequence
EIVLTQSPATLSLSPGERATLSCKASQNVYKWLDWYQQKPGQAPRLLIYNAYSLATGIPARFSGSGSGRDFTLTISSLEPEDFAVYYCQQHNSGWTFGGGTKVEIK

SEQ ID NO: 157 - protein, 106 aa, artificial sequence
  Anti-PAR-2 antibody (P24E889,P24E914,P24E918,P24E922,and P24E932) Variable Light Chain Sequence
EIVLTQSPATLSLSPGERATLSCRASQNIYKWLDWYQQKPGQAPRLLIYNAYSLATGIPARFSGSGSGRDFTLTISSLEPEDFAVYYCQQHNSGWTFGGGTKVEIK

SEQ ID NO: 158 - protein, 106 aa, artificial sequence
  Anti-PAR-2 antibody (P24E930, P24E933, and P24E933) Variable Light Chain Sequence
EIVLTQSPATLSLSPGERATLSCRASQNVYKWLDWYQQKPGQAPRLLIYNAYSRATGIPARFSGSGSGRDFTLTISSLEPEDFAVYYCQQHGSGWTFGGGTKVEIK

SEQ ID NO: 159 - protein, 106 aa, artificial sequence
  Anti-PAR-2 antibody P24E953 Variable Light Chain Sequence)
EIVLTQSPATLSLSPGERATLSCRASQNVYKWLDWYQQKPGQAPRLLIYDAYSRATGIPARFSGSGSGRDFTLTISSLEPEDFAVYYCQQHGSGWTFGGGTKVEIK

SEQ ID NO: 160 - protein, 106 aa, artificial sequence
  Anti-PAR-2 antibody (P24E935,P24E972,and P24E975) Variable Light Chain Sequence
EIVLTQSPATLSLSPGERATLSCRASQNVYKWLDWYQQKPGQAPRLLIYNAYSRATGIPARFSGSGSGRDFTLTISSLEPEDFAVYYCQQHHHGWTFGGGTKVEIK

SEQ ID NO: 161 - protein, 106 aa, artificial sequence
  Anti-PAR-2 antibody P24E977 Variable Light Chain Sequence
EIVLTQSPATLSLSPGERATLSCRASQNVYKWLDWYQQKPGQAPRLLIYDAYSRATGIPARFSGSGSGRDFTLTISSLEPEDFAVYYCQQHHSGWTFGGGTKVEIK

SEQ ID NO: 162 - protein, 106 aa, artificial sequence
  Anti-PAR-2 antibody P24E978 Variable Light Chain Sequence
EIVLTQSPATLSLSPGERATLSCRASQNVYKWLDWYQQKPGQAPRLLIYDAYSRATGIPARFSGSGSGRDFTLTISSLEPEDFAVYYCQQHHHGWTFGGGTKVEIK